European Patent Application EP 4 549 456 A1, published May 7, 2025. Title: RECOMBINANT TYPE-III COLLAGEN AND METHOD FOR PREPARING SAME. Applicant: Bloomage Biotechnology Corporation Limited. The sequence listing filed with the application follows.

SEQUENCE LISTING (6 sequences)

SEQ ID NO: 1 - protein, 449 aa, synthetic construct
EKGETGAPGLKGENGLPGENGAPGAPGERGRPGLPGAAGARGNDGARGSDGQPGPPGPPGTAGFPGSPGAKGEVGPAGSPGSNGAPGQRGEPGPQGHAGAQGPPGPPGINGSPGGKGEMGPAGIPGAPGLMGARGPPGPAGANGAPGLRGGAGEPGKNGAKGEPGPRGERGIPGVPGAKGEDGKDGSPGEPGANGLPGAAGERGAPGFRGPAGPNGIPGEKGPAGERGAPGPAGPRGAAGEPGRDGVPGGPGMRGMPGSPGGPGSDGKPGPPGSQGESGRPGPPGPSGPRGQPGVMGFPGPKGNDGAPGKNGERGGPGGPGPQGPPGKNGETGPQGPPGPTGPGGDKGDTGPPGPQGLQGLPGTGGPPGENGKPGEPGPKGDAGAPGAPGGKGDAGAPGERGPPGLAGAPGLRGGAGPPGPEGGKGAAGPPGPPGAAGTPGLQGMPGER

SEQ ID NO: 2 - protein, 418 aa, synthetic construct
GFPEKGETGAPGAPGAAGARGARGQPGPPGPPGTAGFPGSPGAPGQRGEPGPQGHAGEPGAKGEDGKDGSPGEPGANGEKGPAGAPGPAGPRGAAGEPGRDGGPGMRGMPGSPGGPGSDGKPGPPGSQGESGRPGGPGGPGPQGPPGKNGETGPQGPPGPTGPGGDKGDTGPPGPQGENGKPGEPGPKGDAGAPGAPGGKGDAGPPGLAGAAGTPGLQGDKGEGGAPGPRGSPGETGPPGQNGEPGGKGAPGEKGEGGPQGVKGNPGPPGPSGSPGKDGPPGPAGNTGAPGSPGPKGDAGQPGEKGSPGAQGARGPRGSPGPQGESGKPGPPGPQGTAGEPGRDGNPGSDGRDGSPGGKGDRGENGSPGAPGAPGHPGKSGDRGESGPAGPAGAPGPAGSRGAPGPQGPKGETGAAAP

SEQ ID NO: 3 - protein, 497 aa, synthetic construct
GAPGLKGENGLPGENGAPGAPGERGAAGARGARGQPGPPGPPGTAGAKGSPGAPGQRGEPGPQGHAGEPGPRGERGAKGEDGKDGSPGEPGANGERGEKGPAGERGAPGPAGPRGAAGEPGRDGGPGMRGMPGSPGGPGSDGKPGPPGSQGESGRPGPPGPSGPRGQPGPKGAPGERGGPGGPGPQGPPGKNGETGPQGPPGPTGPGGDKGDTGPPGPQGENGKPGEPGPKGDAGAPGAPGGKGDAGAPGERPPGPEGGKGERGDKGEGGAPGPRGSPGERGETGPPGQNGEPGGKGERGAPGEKGEGGPQGVKGERGARGNPGPPGPSGSPGKDGPPGPAGNTGAPGSPGPKGDAGQPGEKGSPGAQGARGPRGSPGPQGESGKPGERGPPGPQGTAGEPGRDGNPGSDGRDGSPGGKGDRGENGSPGAPGAPGHPGKSGDRGESGPAGPAGAPGPAGSRGAPGPQGPRGDKGETGERGAAGIKGHRGFPGNPGAP

SEQ ID NO: 4 - DNA, 1347 bp, synthetic construct
  source 1..1347: mol_type = other DNA
gaaaagggagaaactggtgccccgggacttaagggagagaacggcctacccggtgaaaatggagcccccggtgctccaggagagcgaggccgccctgggttgccgggcgccgccggtgcccgtgggaatgatggcgccagaggttcggatggacagcctggtccgcccggaccgcctggcactgcgggttttcctgggtctccgggtgcaaaaggagaagtaggaccggctggttcccctggttccaacggggctcccggacaacggggtgaacctggaccacagggtcacgcgggcgcccaggggcctccaggaccaccaggaatcaacggatctccgggtgggaaaggagagatgggccccgcaggtatccctggcgccccaggactgatgggcgcaagggggccgccggggcccgcaggtgcgaatggcgcaccaggactcagaggtggggcaggagagccaggtaagaatggtgctaagggagaacctggtccaaggggagaacgagggattccgggtgtcccgggtgctaaaggcgaggatggcaaagatgggtccccgggagagcccggggcaaatggcctgcccggagcggccggtgaacggggggctccaggtttccgcggacctgcgggtcccaacggtattcctggcgagaaaggacccgctggggaacgtggtgccccggggcccgcgggaccacggggcgccgcaggggaaccagggagggatggtgtccctggtggtcccggcatgaggggaatgcctggttcacctggaggtcccgggtcagatggcaaaccaggaccccctgggagtcaaggcgagagtgggcgcccaggcccccccggcccatctggccctcgtgggcaacctggcgtaatgggatttcccggtccaaagggaaacgacggggcaccgggaaaaaatggggagcgcggggggccagggggccccggtccgcagggtccaccggggaagaacggcgaaactggaccccagggtccccctggaccgaccggcccaggaggcgataaaggtgacacggggccgcctggaccgcaagggcttcaaggattacctggaacaggtggtccaccaggggaaaatggtaaacctggggagccgggaccgaaaggagatgccggcgcaccgggtgctccgggcgggaaaggcgacgcgggcgctccaggtgaacgcgggccaccggggctggccggtgcacccgggctaagaggcggggcgggcccccctggccccgagggaggcaaaggagcggctggcccgcctgggcctcccggcgctgcagggacacccggcctccagggtatgccaggagagcga

SEQ ID NO: 5 - DNA, 1254 bp, synthetic construct
  source 1..1254: mol_type = other DNA
ggtttccccgagaaaggcgaaaccggagcaccgggggccccgggagctgcgggcgctaggggcgctcgtggccaaccaggaccgccggggccgcccggcacagctggatttccaggttcgccgggtgcgccaggtcaacgaggcgaacccggcccccaggggcatgcaggtgagccaggggctaagggggaagatgggaaggacgggtcacccggagaacctggggccaacggggaaaagggaccggcgggggctccagggcccgctggaccgcgtggggcggcgggagaacccggtagggacggcggtccgggcatgcgaggcatgcccggttctccgggtgggcctggcagtgatggtaaacccggcccaccaggttctcaaggagagtccggccggcctggcgggccagggggacctgggcctcagggccccccaggcaaaaatggggagacaggcccccaaggcccaccggggccgacgggtcccggtggtgataaaggagatactggtccgcccgggccacagggtgagaatggtaaacctggtgaaccaggcccaaagggagatgcgggggcgccaggggcgccaggaggtaagggcgatgcaggtcctcccggtctggcgggtgcagcaggcacacccggactccaaggcgacaaaggagaggggggggcaccgggcccaagagggtcgccgggggagacgggacctccgggtcagaatggcgagcctgggggaaagggggccccaggtgagaaaggagaggggggtccacagggcgtaaagggtaaccccggccctccggggccttctggctctccgggaaaagacggcccgccgggaccagccgggaataccggtgctcctgggagccctggaccaaaaggtgacgctggccaacccggagaaaagggcagccctggagcacaaggggctagagggccccggggttcaccgggaccacagggtgaatccggaaaacccggaccgcccggccctcaaggtactgccggcgaacctgggcgcgacggtaaccctggttccgatggccgggacggatcgccgggaggtaaaggcgatcgcggagaaaacggtagtcctggtgcccctggagccccaggccaccccgggaagagtggagaccgtggagagagcggacctgccggccctgcaggagcacccggacctgccggttcaaggggtgcccctggcccacaggggccgaagggggagacgggagcagcggctcct

SEQ ID NO: 6 - DNA, 1491 bp, synthetic construct
  source 1..1491: mol_type = other DNA
ggggcaccgggcctcaaaggagaaaacggtttacctggagaaaatggagcacccggcgcgcccggcgagcgcggagctgcgggtgctcgaggggcacgaggccaacccggaccgcctggtcccccgggaacggctggcgcgaagggatcccctggggcacccgggcagaggggggaaccaggcccgcaggggcacgctggagagcctggccccaggggcgagcggggtgcaaagggagaggatggcaaagatggcagtcccggggagccaggggctaatggagagagaggagagaagggcccagccggtgaaagaggggcccccggccctgcaggtccccgcggggctgccggtgaacccgggcgtgatggtggtcccggcatgagaggcatgcccggttcaccgggtggtccgggttctgacggaaaacccggaccgcccggatctcagggagagtcaggtcgtcctggtccgccagggccctcgggaccgcgaggccagccgggtcctaaaggagcccccggtgagcgcggcggtcctggtgggcctggaccacaaggtcccccaggtaagaatggtgagacaggaccccagggcccgcctggccccaccgggcctgggggcgacaagggggataccggccctccgggtccgcaaggggagaatggtaaaccaggggagccaggcccaaaaggcgacgctggtgctcctggcgctcccggtggcaagggcgacgcaggcgccccaggggagcgtccaccaggacctgaaggggggaaaggagaacggggtgataagggggaaggcggcgcgccaggtcctaggggtagcccgggagaaagaggcgaaactggtccaccaggacaaaacggggaaccaggcgggaaaggcgaaaggggtgcgccaggagaaaagggcgaggggggtcctcagggggttaaaggggagcggggggcccgcgggaaccccggacctccaggacctagtggatcgcccgggaaggacggaccacctgggcctgccgggaatacgggtgcacctggatcaccagggccgaaaggggatgccggccaacccggtgaaaagggttccccaggtgcgcaaggagcccgtggcccgcgggggtctccgggcccgcagggagagtcgggaaagccaggagaacgtggaccgcctgggccacagggaacagcgggagagccgggtcgagacggaaacccaggatctgatgggcgagacggcagccctggtgggaaaggagacagaggagaaaatggcagtcctggagccccgggcgctcccggccatcctggaaagagcggggatagaggagaaagcgggcctgcgggtccggcaggcgctccgggtcccgccggttcccgcggggcaccaggtccgcaagggccacggggcgacaagggagagactggtgaaaggggggcagcgggtattaaagggcatcgaggcttccccggcaacccgggcgcgccc